European Patent Application EP 4 748 392 A1, published May 27, 2026. Title: VACCINE FORMULATION. Applicant: MINERVAX APS. The sequence listing filed with the application follows.

SEQUENCE LISTING (7 sequences)

SEQ ID NO: 1 - protein, 175 aa, synthetic construct
MAEVISGSAVTLNTNMTKNVQNGRAYIDLYDVKNGKIDPLQLITLNSPDLKAQYVIRQGGNYFTQPSELTTVGAASINYTVLKTDGSPHTKPDGQVDIINVSLTIYNSSALRDKIDEVKKKAEDPKWDEGSRDKVLISLDDIKTDIDNNPKTQSDIANKITEVTNLEKILVPRIP

SEQ ID NO: 2 - protein, 170 aa, synthetic construct
STIPGSAATLNTSITKNIQNGNAYIDLYDVKLGKIDPLQLIVLEQGFTAKYVFRQGTKYYGDVSQLQSTGRASLTYNIFGEDGLPHVKTDGQIDIVSVALTIYDSTTLRDKIEEVRTNANDPKWTEESRTEVLTGLDTIKTDIDNNPKTQTDIDSKIVEVNELEKLLVLS

SEQ ID NO: 3 - protein, 347 aa, synthetic construct
MAEVISGSAVTLNTNMTKNVQNGRAYIDLYDVKNGKIDPLQLITLNSPDLKAQYVIRQGGNYFTQPSELTTVGAASINYTVLKTDGSPHTKPDGQVDIINVSLTIYNSSALRDKIDEVKKKAEDPKWDEGSRDKVLISLDDIKTDIDNNPKTQSDIANKITEVTNLEKILVPRIPEFSTIPGSAATLNTSITKNIQNGNAYIDLYDVKLGKIDPLQLIVLEQGFTAKYVFRQGTKYYGDVSQLQSTGRASLTYNIFGEDGLPHVKTDGQIDIVSVALTIYDSTTLRDKIEEVRTNANDPKWTEESRTEVLTGLDTIKTDIDNNPKTQTDIDSKIVEVNELEKLLVLS

SEQ ID NO: 4 - protein, 173 aa, synthetic construct
MAEVISGSAATLNSALVKNVSGGKAYIDIYDVKNGKIDPLNLIVLTPSNYSANYYIKQGGRIFTSVNQLQTPGTATITYNILDENGNPYTKSDGQIDIVSLVTTVYDTTELRNNINKVIENANDPKWSDDSRKDVLSKIEVIKNDIDNNPKTQSDIDNKIVEVNELEKLLVLP

SEQ ID NO: 5 - protein, 172 aa, synthetic construct
STIPGSAATLNTSITKNIQNGNAYIDLYDVKNGLIDPQNLIVLNPSSYSANYYIKQGAKYYSNPSEITTTGSATITFNILDETGNPHKKADGQIDIVSVNLTIYDSTALRNRIDEVINNANDPKWSDGSRDEVLTGLEKIKKDIDNNPKTQIDIDNKINEVNEIEKLLVVSL

SEQ ID NO: 6 - protein, 347 aa, synthetic construct
MAEVISGSAATLNSALVKNVSGGKAYIDIYDVKNGKIDPLNLIVLTPSNYSANYYIKQGGRIFTSVNQLQTPGTATITYNILDENGNPYTKSDGQIDIVSLVTTVYDTTELRNNINKVIENANDPKWSDDSRKDVLSKIEVIKNDIDNNPKTQSDIDNKIVEVNELEKLLVLPEFSTIPGSAATLNTSITKNIQNGNAYIDLYDVKNGLIDPQNLIVLNPSSYSANYYIKQGAKYYSNPSEITTTGSATITFNILDETGNPHKKADGQIDIVSVNLTIYDSTALRNRIDEVINNANDPKWSDGSRDEVLTGLEKIKKDIDNNPKTQIDIDNKINEVNEIEKLLVVSL

SEQ ID NO: 7 - protein, 103 aa, synthetic construct
VVEGSAATLNTAMTKNMQNGNAYIDIYDVKLGKIDPLQLIKLEPGYTAIYYITQGSKVYANVSELQTPGAAKVNYRIQTSDGSDHIKSDGQLDSVNISLTVYD